European Patent Application EP 4 317 191 A1, published February 7, 2024. Title: Improved  nicotinamide phosphoribosyltransferase. Applicant: Mitsubishi Chemical Corporation. The sequence listing filed with the application follows.

SEQUENCE LISTING (50 sequences)

SEQ ID NO: 1 - protein, 11 aa, Artificial Sequence
  motif sequence
  MISC_FEATURE (2)..(2): Xaa stands for Val or Ile
  MISC_FEATURE (5)..(6): Xaa can be any naturally occurring amino acid
  MISC_FEATURE (9)..(9): Xaa stands for Thr, Val, or Ile
  MISC_FEATURE (10)..(10): Xaa stands for Met, Val, or Ile
  MISC_FEATURE (11)..(11): Xaa can be any naturally occurring amino acid
SXPAXXHSXXX

SEQ ID NO: 2 - protein, 4 aa, Artificial Sequence
  motif sequence
  MISC_FEATURE (1)..(1): Xaa can be any naturally occurring amino acid
  MISC_FEATURE (2)..(2): Xaa stands for Ser or Ile
  MISC_FEATURE (4)..(4): Xaa can be any naturally occurring amino acid
XXDX

SEQ ID NO: 3 - protein, 501 aa, Haemophilus ducreyi
MDNLLNYSSRASAIPSLLCDFYKTSHRIMYPECSQIIYSTFTPRSNEQAPYLTQVVSFGFQAFIIKYLIHYFNDNFFSRDKHDVVTEYSAFIEKTLQLEDTGEHIAKLHELGYLPIRIKAIPEGKTVAIKVPVMTIENTHSDFFWLTNYLETLINVSLWQPMTSASIAFAYRTALIKFANETCDNQEHVPFQSHDFSMRGMSSLESAETSGAGHLTSFLGTDTIPALSFVEAYYGSSSLIGTSIPASEHSVMSSHGVDELSTFRYLMAKFPHNMLSIVSDTTDFWHNITVNLPLLKQEIIARPENARLVIRPDSGNFFAIICGDPTADTEHERKGLIECLWDIFGGTVNQKGYKVINPHIGAIYGDGVTYEKMFKILEGLQAKGFASSNIVFGVGAQTYQRNTRDTLGFALKATSITINGEEKAIFKNPKTDDGFKKSQKGRVKVLSRDTYVDGLTSADDFSDDLLELLFEDGKLLRQTDFDEIRQNLLVSRTTLHHHHHH

SEQ ID NO: 4 - DNA, 1506 bp, Haemophilus ducreyi
atggacaatctgctgaactactcctcacgcgcctcggcaatcccgtccctgctgtgcgacttctacaaaacctctcatcgtattatgtatccggaatgctctcagattatctatagtacctttacgccgcgttcgaacgaacaggcaccgtacctgacccaagtggttagcttcggcttccaagctttcatcatcaaatacctgatccattacttcaacgataactttttcagccgtgataaacacgacgtcgtgaccgaatatagtgcgtttattgaaaaaaccctgcagctggaagacacgggcgaacatatcgccaaactgcacgaactgggttacctgccgattcgtatcaaagcaattccggaaggtaaaaccgttgctattaaagttccggtcatgaccatcgaaaatacgcattctgatttcttttggctgaccaactatctggaaacgctgatcaatgtcagtctgtggcagccgatgaccagcgcgtcaattgcgtttgcctaccgtaccgcactgatcaaattcgctaacgaaacgtgtgataatcaggaacatgtgccgtttcaatcccacgacttctcaatgcgcggcatgagctctctggaatcggcggaaaccagcggcgccggtcatctgacgtcctttctgggtaccgatacgattccggcgctgtcattcgttgaagcctattacggcagttcctcactgattggtaccagcatcccggcatcggaacatagcgttatgtcgagccacggcgtcgatgaactgagcacgtttcgctatctgatggctaaattcccgcataacatgctgtctattgtcagtgataccacggacttttggcacaacatcaccgtgaatctgccgctgctgaaacaggaaattatcgcacgtccggaaaacgctcgtctggtgattcgcccggatagcggcaactttttcgcgattatctgcggtgatccgaccgccgacacggaacatgaacgcaaaggtctgattgaatgtctgtgggatatctttggcggtaccgtgaaccagaaaggctataaagttatcaatccgcacattggtgcaatctatggcgacggtgttacgtacgaaaaaatgttcaaaatcctggaaggcctgcaagcgaaaggttttgcctctagtaacatcgtcttcggcgtgggtgcgcagacctaccaacgtaatacccgcgatacgctgggctttgcactgaaagctaccagcattacgatcaacggtgaagaaaaagccatcttcaaaaacccgaaaaccgatgacggcttcaaaaaatcgcagaaaggtcgtgtgaaagttctgagccgcgatacctatgtggacggcctgacgtccgccgatgacttttcagatgacctgctggaactgctgttcgaagatggtaaactgctgcgtcagaccgactttgatgaaatccgtcagaacctgctggttagccgcacgaccctgcaccaccaccaccaccactga

SEQ ID NO: 5 - protein, 463 aa, Meiothermus ruber
MKTLNPHNLILNTDSYKASHFAQFPKGMTYASWYIESRGGDSNFVRFFGLQAFLIEYLSKGVSLADVEEAQEVFLAHGLPFPTEGWRYIAQDLGGRLPVRIRAVPEGKVVPVHNPLVIIESTDPKVPWLPGWLETALLRAVWYPTTVCTVSWGIRNTIKEYLEKTADDPEAELPFKLHDFGARGVSSLESAGLGGMAHLVNFMGTDTVTALIYARNYYGAEMAGYSIPAMEHSTVTSFGRTGEAQAYRQMLETFAKPGALMAMVIDSYNREHAVGQIIGEELRELIQQSGATVVIRPDSGDPPFVVLRTVQTLEAKFGATLNRKGYKVLNGVRVIQGDGVNADSIRKVLFLLEQWGYSASNVAFGMGGALLQHPHRDTQKFAQKLHLVTVNGETYGVGKSPVDDPGKLSKKGRLDVIQDERGIRTVELPLEAAQPHPQSILQTVFENGSITRRYTWEEVRNNA

SEQ ID NO: 6 - DNA, 1389 bp, Meiothermus ruber
atgaaaaccctgaatccgcataacctgatcctgaataccgatagctacaaagcgagccacttcgcgcagttcccgaaaggcatgacctacgcgagctggtacatcgaaagccgtggtggcgacagcaacttcgtgcgtttctttggtctgcaggcgtttctgattgagtatctgagcaagggcgtgagcctggcggatgttgaggaagcgcaagaggttttcctggcgcacggtctgccgtttccgaccgaaggctggcgttacattgcgcaggacctgggtggccgtctgccggtgcgtattcgtgcggttccggagggcaaggtggttccggtgcacaacccgctggttatcattgaaagcaccgatccgaaagttccgtggctgccgggttggctggaaaccgcgctgctgcgtgcggtttggtacccgaccaccgtgtgcaccgttagctggggcatccgtaacaccattaaggagtatctggaaaaaaccgcggatgatccggaggcggaactgccgttcaagctgcacgactttggtgcgcgtggcgtgagcagcctggaaagcgcgggtctgggtggcatggcgcacctggtgaacttcatgggcaccgataccgttaccgcgctgatctacgcgcgtaactactatggtgcggagatggcgggctatagcattccggcgatggaacacagcaccgttaccagctttggtcgtaccggtgaagcgcaggcgtaccgtcaaatgctggaaacctttgcgaaaccgggtgcgctgatggcgatggtgatcgacagctataaccgtgagcacgcggttggtcaaatcattggcgaggaactgcgtgaactgatccagcaaagcggtgcgaccgtggttattcgtccggacagcggcgatccgccgtttgtggttctgcgtaccgtgcagaccctggaagcgaagtttggtgcgaccctgaaccgtaagggttacaaagttctgaacggcgtgcgtgttatccaaggtgacggcgtgaacgcggatagcattcgtaaagttctgttcctgctggagcagtggggttatagcgcgagcaacgtggcgtttggtatgggtggcgcgctgctgcaacacccgcaccgtgatacccagaagtttgcgcaaaaactgcacctggtgaccgttaacggtgaaacctatggtgtgggcaagagcccggttgacgatccgggtaaactgagcaagaaaggccgtctggacgtgatccaggatgagcgtggcattcgtaccgttgaactgccgctggaagcggcgcagccgcacccgcaaagcatcctgcagaccgtttttgaaaatggcagcatcacccgtcgctatacctgggaagaagttcgtaataatgcg

SEQ ID NO: 7 - protein, 474 aa, Xanthomonas translucens
MQCLNNLLLNTDSYKASHWLQYPAGTDATFFYVESRGGVYDRTVFFGLQSILKEALGRAVTHADIDEARDLFAAHGEPFNEAGWRDIVDRLGGQLPIRIRAVPEGSVVPTHNALMTIESTDAQAYWVPSYLETLLLRIWYPVTVATVSWHAKQTLRQFLERTSDDPEGQLPFKLHDFGARGVSSLESAAIGGAAHLVNFLGTDTVSGLLLARAHYHEPMAGYSIPAAEHSTITSWGREREVDAYRNMLKQFGKPGGIVAVVSDSYDIFHAIREHWGTTLREEVIASGATVVIRPDSGDPVAVVHQCLELLDEAFGHRVNGKGYKVLNHVRVIQGDGVNPTSIRAILERVTSAGYATDNVAFGMGGALLQRLDRDTQKFALKCSAARVDGTWIDVYKDPVTDKGKLSKRGRMSLLRHREYGGYRTEPVPATAASLDALARPTGYDDAMVTVWENGRLLHDWSLAQVRDRANAARL

SEQ ID NO: 8 - DNA, 1422 bp, Xanthomonas translucens
atgcagtgcctgaacaatctgctgctgaacactgattcttataaagcatctcactggctgcagtacccggcaggtactgacgctaccttcttttacgtagaatcccgtggtggcgtttacgatcgtaccgttttttttggtctgcagagcatcctgaaagaagcactgggtcgtgcggttacgcacgctgatatcgatgaagcgcgtgacctgtttgctgcgcacggcgaaccgtttaacgaagcaggttggcgtgacatcgttgaccgtctgggtggccaactgccgattcgtatccgtgcggttccggaaggttccgtggttccgactcacaacgcactgatgactatcgagagcacggacgcacaggcttactgggtgccgtcctatctggagaccctgctgctgcgtatctggtacccggttactgttgcaaccgtgtcttggcacgcgaaacagaccctgcgtcaattcctggaacgtacttccgatgatccggaaggtcagctgccgttcaaactgcatgatttcggtgcacgtggtgtttctagcctggaatctgcagctattggtggcgcggctcatctggttaacttcctgggcactgacaccgtatctggtctgctgctggcacgtgcccattatcacgaaccgatggcgggctatagcattccagcggccgaacacagcaccatcacctcctggggccgcgaacgtgaagttgacgcatatcgcaacatgctgaagcagttcggtaagccgggcggtatcgttgcggtcgtatccgactcttacgacatttttcacgcgatccgcgaacactggggcactaccctgcgcgaagaagtaatcgcatctggtgccaccgttgtgattcgtccggactctggtgatccggttgcggttgtccaccagtgtctggaactgctggatgaagctttcggtcaccgcgtgaacggcaaaggctacaaggtcctgaaccacgtccgtgttatccagggcgacggtgttaacccgaccagcatccgtgcgatcctggagcgtgttacgagcgcaggctacgcgaccgataacgtagctttcggtatgggtggtgctctgctgcaacgtctggatcgtgacacccagaaatttgctctgaagtgttctgcggcacgcgtcgatggcacctggattgacgtgtacaaagatccagtgaccgataaaggtaagctgtctaaacgtggccgtatgtctctgctgcgtcatcgtgaatatggtggttatcgtactgagccagttccagcgactgctgccagcctggatgctctggctcgtccaaccggttacgacgacgcaatggtgaccgtgtgggaaaacggtcgtctgctgcacgattggtctctggcccaggttcgtgatcgtgcaaatgcagcccgtctg

SEQ ID NO: 9 - protein, 461 aa, Sphingopyxis sp. C-1
MKNLILATDSYKQSHFLQYPPEARVISAYVEARPNPFSEEIVFLGLQPLLVDYFSQPINAADIDEAEAICIAHGVPFNRAGWEAIVADHGGYLPLEIKALPEGAIVPAGVPLVQLENTDPRMPWLTTFIETAMLRAIWYPTTVATLSWKCKQVIRAGLEKTSDDVEGQLPFKLHDFGARGVSSAESAGLGGLAHLVNFQGTDTMEALVAARRYYGADMAGFSIPAAEHSTMTSWGRDREEDAYRNMLDRFEGEGRIVAVVSDSYDLDTAVTDIWGGSLREKVLGRAGTLVVRPDSGDPIETPLRTVKTLWEKFGGHVNGKGYRVLDPHVRVIQGDGMTVDSIGRLVQRMIEEGFAIDNIAFGMGGGMLQHVNRDTLRFAMKANAMLGSDGVWHDVFKMPSTDPGKASKAGRQAVVLKDGRMAAARLDSVAVGEDLLVPVWRNGELLVRHDFDAVRKRSEGR

SEQ ID NO: 10 - DNA, 1383 bp, Sphingopyxis sp. C-1
atgaagaatctgattctggccaccgatagctataaacagagccattttctgcagtatccgcctgaagcacgtgttattagcgcatatgttgaagcccgtccgaatccgtttagcgaagaaattgtttttctgggtctgcagccgctgctggttgattatttcagccagccgattaatgcagccgatattgatgaagcagaagccatttgtattgcacatggtgttccgtttaatcgtgcaggttgggaagcaattgttgcagatcatggtggttatctgccgctggaaattaaagcactgccggaaggtgcaattgttccggcaggcgttccgctggttcagctggaaaataccgatccgcgtatgccgtggctgaccacctttattgaaaccgcaatgctgcgtgcaatttggtatccgaccaccgttgcaaccctgagctggaaatgcaaacaggttattcgtgccggtctggaaaaaaccagtgatgatgttgaaggtcagctgccgtttaaactgcatgattttggtgcacgtggtgttagcagcgcagaaagcgcaggtttaggtggtctggcacatctggttaattttcagggcaccgataccatggaagcactggttgcagcccgtcgttattatggtgcagatatggcaggttttagcattccggcagcagaacatagcaccatgaccagctggggtcgtgatcgtgaagaagatgcatatcgtaatatgctggatcgctttgaaggtgaaggtcgtattgttgccgttgttagcgatagttatgatctggataccgcagttaccgatatttggggtggtagcctgcgtgaaaaagttctgggtcgtgcgggtacactggttgttcgtccggatagcggtgatccgattgaaacaccgctgcgtaccgttaaaaccctgtgggaaaaatttggtggtcatgtgaatggtaaaggttatcgtgttctggatccgcatgttcgtgttattcaaggtgatggtatgaccgttgatagcattggtcgtctggtgcagcgtatgattgaagaaggttttgccattgataacattgcctttggtatgggtggtggtatgctgcaacatgttaatcgtgataccctgcgttttgcaatgaaagcaaatgcaatgctgggtagtgatggtgtttggcatgatgtgtttaaaatgccgagcaccgatccgggtaaagcaagcaaagcaggtcgtcaggcagttgttctgaaagatggtcgtatggcagcagcacgtctggatagcgttgcagttggtgaagatctgctggttccggtttggcgtaatggtgaactgctggtgcgtcacgattttgatgcagttcgtaaacgtagcgaaggtcgt

SEQ ID NO: 11 - protein, 471 aa, Chitinophaga pinensis
MTKENLILLADAYKYSHHKLYIPGTEYIYSYFESRGGKFNETVFYGLQYFLMEYLQGAVITKEKLDEAEATLLEVFGRNDVFDRTRFEYIIEKHGGRLPVRIKAVPEGTVTGVRNVLMTIENTDPNCYWVTNFLETLLMQIWYPCTVATLSREIKKTVKQYYNETASEAAFAGIDFVLNDFGFRGASSVESAGIGGSAHLINFSGSDTLIGSTFAKRYYQAPVAPGLSIPATEHSIVTMLGEEGELEIFRHILNAFPTGTIACVSDSYNILRACREYWGTELKEQILSRQGTLVIRPDSGDAIQTLLKVFEILMETFGYTVNEKGYKVLPPQVRVIQGDGISYSSIPPIFEALKQAGISAENLVLGMGGALLQRVNRDTQEYALKCSFAQVNGKAINVQKNPLELDANGNTRVSFKKSKSGKQKLVVENGIYTSLPENEAPALADQLVTVFEDGEIKKAYSFEQIRKNATI

SEQ ID NO: 12 - DNA, 1413 bp, Chitinophaga pinensis
atgaccaaagaaaacctgattctgctggcagatgcatacaaatatagccaccacaaactgtatattccgggaaccgaatatatctacagctattttgaaagccgtggtggcaaatttaacgaaaccgttttttatggcctgcagtacttcctgatggaatatctgcagggtgcagttatcacaaaagaaaaactggatgaagcagaagcaaccctgctggaagtttttggtcgtaatgatgtttttgatcgcacccgctttgaatacatcattgaaaaacatggtggtcgtctgccggttcgtattaaagcagttccggaaggcaccgttaccggtgttcgtaatgttctgatgaccattgaaaataccgatccgaattgttattgggtgaccaattttctggaaacactgctgatgcagatttggtatccgtgtaccgttgcaaccctgagccgtgaaatcaaaaaaaccgttaaacagtattacaatgaaaccgcaagcgaagcagcatttgcaggtattgattttgtgctgaacgattttggttttcgtggtgcaagcagcgttgaaagtgccggtattggtggtagcgcacatctgattaactttagcggtagcgataccctgattggtagcacctttgcaaaacgttattatcaggcaccggttgcaccgggtctgagcattccggcaacagaacattcaattgttaccatgctgggtgaagaaggtgaactggaaatttttcgccatattctgaatgcatttccgaccggcaccattgcatgtgttagcgatagctataacattctgcgtgcatgtcgtgaatattggggcaccgaactgaaagagcagattctgagccgtcagggcaccctggttattcgtccggatagcggtgatgcaattcagacgctgctgaaagtgtttgaaattctgatggaaacctttggctataccgtgaacgaaaaaggctataaagttctgcctccgcaggttcgtgttattcaaggtgatggtattagctatagcagcattccgcctatttttgaagcactgaaacaggcaggtattagcgcagaaaatctggttttaggtatgggtggtgcactgctgcagcgtgttaatcgtgatacccaagaatatgcactgaaatgtagctttgcacaggttaatggcaaagccattaatgtgcagaaaaatccgctggaactggatgcaaatggtaatacccgtgtgagtttcaaaaaaagcaaaagcggtaaacagaaactggtggtggaaaatggtatttataccagcctgccggaaaatgaagcaccggcactggcagatcagctggttaccgtttttgaagatggcgaaattaagaaagcctatagctttgagcagatccgtaaaaacgcaaccatc

SEQ ID NO: 13 - protein, 471 aa, Chitinophaga arvensicola
MTKENLILLADAYKYSHHKLYIPGTQFIYSYLESRGGKFEETVFYGLQYFLKEYLSGVVFTKEKLDEAETMLTEVFGRSDVFDRSRFEYIIDKYGGKLPVRIKAVAEGTVVPVRNVLMTIENTDPECFWLTNFLETLLMQVWYPCTVASVSREIKKVVKQYYEATASQEAFTGIDFVLNDFGFRGASSVESAGIGGSAHLVNFAGSDTIPGSVFAKRYYGATTAPGLSIPATEHSVVTLLGEEGELEIFKHILDTYPTGTIACVSDSYNIFRACEQYWGTELKEQILKREGTLVIRPDSGDPVQTLLRIFNILMDKFGYTTNEKGFKVLPPQVRVIQGDGISYSSIPGIFEALKQAGISAENLVLGMGGALLQRVNRDTQEFALKCAYAVVNGEAINVQKMPVELDATGQLRTSFKKSKAGKLRLIKDNNTFKTVGEGEAPASADLLHTVFENGEVVHSYTFDEVRKTAAL

SEQ ID NO: 14 - DNA, 1413 bp, Chitinophaga arvensicola
atgaccaaggagaacctgatcctgctggctgacgcgtacaaatactcccaccacaaactgtacattccaggcacgcagttcatttactcttacctggaatctcgcggcggcaaattcgaggaaaccgttttttatggcctgcagtactttctgaaggaatacctgagcggcgttgtattcacgaaagaaaagctggatgaagctgaaacgatgctgaccgaggtattcggccgctccgatgtattcgatcgctcccgtttcgaatatatcatcgataagtacggtggtaagctgccggtgcgcatcaaggcggtcgctgaaggtactgtggtgcctgttcgcaacgttctgatgaccatcgaaaacaccgatcctgaatgcttttggctgactaactttctggaaaccctgctgatgcaggtgtggtatccatgcactgtggcatctgtaagccgcgaaatcaaaaaagtggtgaaacagtactacgaggctacggccagccaggaagcattcaccggtatcgacttcgtactgaacgattttggcttccgtggcgcctcctctgtggaatctgcaggtattggtggttccgcacatctggttaattttgccggctccgataccatcccaggctctgttttcgctaaacgttattatggtgctaccaccgctccgggtctgtctattccggctactgaacactccgtggttacgctgctgggcgaagagggtgaactggaaatcttcaagcacatcctggatacctatccgactggtactatcgcttgcgtgtccgacagctacaacatctttcgtgcgtgtgaacaatactggggtaccgaactgaaagaacagatcctgaagcgcgaaggcaccctggtaatccgtcctgattctggcgacccggttcagactctgctgcgtatcttcaacatcctgatggacaagttcggttacaccactaacgaaaaaggcttcaaagtactgccgccacaggtacgcgtgatccagggtgacggtatcagctacagcagcatcccgggcatctttgaggcactgaaacaggctggcatcagcgctgaaaacctggtactgggcatgggtggtgcactgctgcagcgtgtcaatcgtgatacccaagagttcgccctgaaatgcgcatacgcagttgtcaatggtgaggccatcaacgtccagaaaatgccagtagaactggatgcaaccggtcagctgcgtacctccttcaaaaaatccaaagcaggtaagctgcgcctgatcaaagataacaataccttcaagaccgtgggtgaaggcgaagcacctgcgtctgcagacctgctgcatacggtcttcgagaacggtgaggttgtgcattcctacacctttgacgaagtacgtaaaaccgctgcactg

SEQ ID NO: 15 - protein, 477 aa, Burkholderia pyrrocinia
MQNDPGGFAAVLANPILNTDSYKASHFLQYPPDASAMFSYVESRGGRYDRTLFFGLQMLLKEYLCKPVTHAMIDDARDFFTVHGVPFNEAGWRYIVERYDGYLPVKIRAVPEGSVVPVHNVLMTVECDDPQVFWLASYLETMLLRVWYPVTVATRSWHLRQTIRRFLERTDDDLAQLPFKLHDFGARGVSSAESAAIGGAAHLVSFMGSDTVLGVLAANRFYREPMAAYSVPAAEHSTITSWGREGEADAYRNMIRRFGLPGAIVSVVSDSYDLFAALDLWGGELRQAVIDSGATLVVRPDSGDPVKIVMQTVRALDVSFGSTLNGKGRRVLNRVRVIQGDGVDELSIDAILSALDDAGYAAGNVVFGMGGALLQQVNRDTQRFAMKCSAIRRDGVWHDVRKDPVTDQGKRSKKGRLTLLRNRRTGEYRTTTLPVAWDDRALEGEWDEALETVFDTGRLLVDTTFAEVRARAHAGEV

SEQ ID NO: 16 - DNA, 1431 bp, Burkholderia pyrrocinia
atgcagaatgatccaggcggttttgctgcagttctggctaaccctatcctgaacaccgactcctacaaagcatcccattttctgcaatacccgcctgacgcctctgcgatgttctcctacgttgaatcccgtggcggtcgttatgaccgtaccctgttcttcggtctgcagatgctgctgaaggaatacctgtgtaaaccggtgactcacgcgatgattgatgatgcgcgtgacttctttaccgtacacggtgtgcctttcaacgaagcaggttggcgctatatcgttgaacgttatgatggctacctgcctgtaaagatccgcgctgttccagaaggcagcgttgtaccggtccacaacgtactgatgaccgttgaatgtgatgatccgcaggtattctggctggctagctacctggaaactatgctgctgcgtgtttggtatcctgttactgtcgcgacccgttcctggcatctgcgtcaaactatccgccgtttcctggagcgtaccgatgacgacctggcgcaactgccgtttaaactgcacgactttggcgctcgtggtgtttcctccgcggaatctgctgccattggtggtgctgcgcatctggtttcctttatgggcagcgatactgtactgggtgtcctggctgctaaccgtttttaccgtgaaccgatggcagcgtattctgtaccagccgctgaacactccaccatcacctcttggggtcgtgaaggtgaagctgatgcctaccgtaacatgatccgtcgtttcggcctgccgggtgctattgtctccgtagtctctgactcttatgacctgttcgctgctctggatctgtggggtggtgaactgcgtcaggctgtgatcgattccggcgcgaccctggttgttcgtccggattccggtgacccagtgaaaattgtgatgcagactgtgcgtgcgctggacgtttctttcggttccacgctgaacggtaaaggtcgccgtgtgctgaaccgtgtgcgtgtgattcagggcgacggcgttgatgaactgagcatcgacgctatcctgtctgcactggacgatgcgggttatgcggcaggcaacgttgtgttcggtatgggtggcgccctgctgcagcaagtcaaccgtgacacccaacgttttgcaatgaaatgctccgcgatccgtcgcgacggtgtatggcacgacgtacgtaaagatccggtcaccgaccagggcaagcgctctaaaaaaggtcgtctgacgctgctgcgtaaccgtcgcactggtgaatatcgcaccaccactctgccggttgcttgggatgaccgtgctctggagggtgaatgggacgaagcgctggaaactgtttttgacactggtcgcctgctggtagatacgaccttcgcggaagttcgtgcacgtgcacatgctggtgaagtg

SEQ ID NO: 17 - protein, 485 aa, Pedobacter alluvionis
MNPLLLTDGYKVDHRRQYPENTTLVYSNWTPRKSRLENVNHVVLFGLQYFIKKYIIEDFNQNFFKQPKEEILKKYARRINNYLGENLVGTQHIADLHDLGYIPMVFKSLPEGAEVPLRVPMFTMYNTKPEFFWLTNYFETLLSAVVWLPCNSATIAKQYRTILDRYAAETSSVPEFVDWQGHDFSMRGMGGIEAAVTSAAGHLLSFTGTDTIPAIDFLEEYYNADSDKELIGGSVAATEHSVMCMGTNTGELETFKRLILEVYPKGIVSIVSDTWDLWKVLTEYLPILKDDIIARPGKVVIRPDSGDPVDIICGNPDGKSENEKKGVIELLWDVFGGKTNDKGFKELVPQIGAIYGDSITTERATQICERLKAKGFASTNVVFGIGSFTYQYNTRDTFGFAMKATYGEVDGEGREIFKDPITDDGTKKSAKGLLQIFKNASGDYELKDQCTWEEEAQGELKEVFRDGKLLIDYSLAEIRERLKNS

SEQ ID NO: 18 - DNA, 1455 bp, Pedobacter alluvionis
atgaatccgctgctgctgactgatggctacaaagtcgatcaccgccgccagtacccggaaaacacgacgctggtatatagcaactggaccccgcgcaaatcccgtctggagaacgttaatcacgtcgttctgtttggcctgcagtatttcatcaaaaaatacatcatcgaagactttaaccaaaactttttcaaacagccgaaggaagaaattctgaaaaaatacgctcgtcgtatcaacaactacctgggtgaaaatctggtgggtacccagcacatcgcagacctgcacgacctgggttacattccgatggtgttcaaatctctgccagaaggtgcggaagtgcctctgcgtgtgccgatgttcacgatgtacaacaccaaacctgaattcttctggctgaccaactacttcgaaaccctgctgtccgctgttgtttggctgccgtgcaactctgcgaccatcgcaaaacagtatcgtaccatcctggatcgctatgccgcagagacctctagcgttccggaattcgtggattggcagggtcacgacttctctatgcgtggcatgggcggtattgaagcagcggtaacctctgcagcgggccatctgctgtcctttactggcaccgacacgattccagccattgactttctggaagaatactataacgcagacagcgataaagaactgattggcggctccgttgctgcaactgaacactccgtcatgtgtatgggtaccaacactggtgaactggaaaccttcaaacgtctgatcctggaggtttatccaaaaggtatcgtgtctattgtatctgatacttgggacctgtggaaagtgctgacggaatatctgccgattctgaaggatgatatcattgcccgcccaggcaaagttgtgatccgtccggatagcggtgacccggtcgatatcatttgcggcaacccggacggtaaatctgaaaacgaaaagaagggcgttatcgagctgctgtgggatgttttcggcggtaaaaccaacgacaaaggttttaaagagctggtaccacagatcggcgctatctatggcgattccatcaccactgaacgcgcgacccagatctgtgaacgcctgaaagcaaaaggttttgcttccactaacgtagtttttggtatcggcagcttcacttaccagtacaacacccgcgacaccttcggtttcgcaatgaaagcgacgtatggcgaagtagatggtgaaggccgtgagatctttaaagatccgattaccgatgacggcaccaaaaaatctgctaaaggtctgctgcagatcttcaagaacgcttctggtgactatgaactgaaagaccaatgcacctgggaagaagaggcgcagggcgaactgaaggaggtgttccgtgacggcaaactgctgatcgattactctctggcagaaattcgcgagcgtctgaaaaactct

SEQ ID NO: 19 - protein, 473 aa, Microbulbifer thermotolerans
MQDYNPILNVDSYKTSHYLQYPEGTQYVSSYIESRGGQFKEAVFFGLQAFITQYLSQPITRNDIEEAEELCLAHGVPFNRAGWEYILEAHQGYLPIEIQAVPEGTVVPVQNVLAQVVNTDPKCFWITSYVETALLRAIWYPTTVATQSREAKKIIQRYLEETADTLDGLPFKLHDFGARGASSGETAALGGLAHLVNFQGTDTVAALVAGRRFYNAPMAGFSIPAAEHSTMTSWGREHETEAYANMLTQFAGDGRVVAVVSDSYNLWNAIDNIWGGELKERVENNGGTLVIRPDSGDPVDVVTQTIERLMRIFGARINSKGYRVLPDYIRVIQGDGISLHTIEGILAAMKARKQSADNIAFGMGAELLQKVHRDTMKFAMKASAVRVNGLWRDVFKDPVTDTGKRSKKGRLALIRRGNGELRTIREQDLGNRQNLLQPVFRNGKLLTEQSLEDIRRRAAVPHNEDELVMAAVS

SEQ ID NO: 20 - DNA, 1419 bp, Microbulbifer thermotolerans
atgcaggactacaacccgatcctgaacgtagattcctacaaaaccagccattacctgcagtatccagagggcacccagtacgtttcttcttatatcgaatcccgtggcggtcagttcaaagaagctgtgttttttggtctgcaggcgttcatcacccagtacctgagccagccaatcacccgcaatgacatcgaagaggctgaagaactgtgcctggcacacggtgttccgttcaaccgtgcaggttgggaatatatcctggaggcgcaccagggctatctgccgatcgaaatccaagccgtgccggaaggcaccgttgtcccggtgcagaacgttctggcgcaggtagttaacactgatccgaaatgcttttggatcaccagctacgtagaaacggcactgctgcgcgcgatctggtacccgactactgtggcgacccagagccgcgaggctaagaagatcattcaacgttacctggaagagactgcagacaccctggatggtctgccttttaaactgcacgacttcggcgcgcgtggcgcatcttctggcgaaacggcggccctgggtggtctggctcacctggtcaacttccaaggtaccgatacggttgcggcactggttgcgggccgtcgtttttataacgcgccaatggctggtttttccatcccagcagctgagcactctactatgaccagctggggccgcgagcacgaaaccgaggcctacgcaaacatgctgacccagtttgctggcgatggtcgtgtggttgctgtggtgtctgactcctacaacctgtggaacgctatcgacaatatttggggcggtgaactgaaagagcgcgtggaaaacaacggcggtaccctggtaatccgtccggatagcggcgatccagttgatgtagttacccagactatcgaacgtctgatgcgtattttcggcgctcgcatcaactctaaaggttatcgcgtcctgccggactacatccgtgtgatccagggtgacggtatctctctgcacactatcgagggcatcctggcggcaatgaaggcccgcaaacagagcgcagataacattgcttttggcatgggcgctgaactgctgcaaaaagtgcaccgcgataccatgaaattcgcgatgaaagcatccgccgtacgcgttaacggcctgtggcgtgatgtgttcaaagatccggttactgataccggtaaacgttctaagaagggccgtctggcactgatccgtcgcggcaacggcgaactgcgtaccatccgtgaacaggatctgggtaaccgccaaaacctgctgcagccagttttccgcaacggtaagctgctgaccgaacagtccctggaggatattcgtcgtcgtgcggcggttccacacaacgaggatgaactggtgatggcggctgtctcc

SEQ ID NO: 21 - protein, 468 aa, Labrenzia aggregata
MTNPLLATDSYKQSHFKQYPPEARRISAYLEARPNPFSDSVLFFGLQTYLKDVLLKPITASDIAAADRICAAHGVPFNREGWEQILTDHGGLFPLEIKALPEGTLAPSGVPLVQVENTDERMPWLTTWVETALLRSVWYPSTVATLSFKCKEILYRGLLDTSDDPDSQIPFKLHDFGARGVSSAESAALGGMAHLVNFAGTDTMEALEAAMTWYGADVAGFSIPAAEHSTMTSWGREREVDAYRNMLVQFGRPNAPVAVVSDSYDLGNAVENLWCGRLKDEVLKSGATVVIRPDSGDPVEMPLKVMETLWQHYGGSENSKGARVLHPSVRVIQGDGMKLDTIRQLVEELVRRNWSVDNIAVGMGGGLLQQVNRDTMRFAMKANAMKTADGTWHDVSKNPATDPGKASKAGRQATVLENGVLSAVRLEAVGGRTDQLQTVYRNGVLVKDWTFEEVRALARKHLLERVAS

SEQ ID NO: 22 - DNA, 1404 bp, Labrenzia aggregata
atgactaacccactgctggcgactgattcttacaaacagagccacttcaaacagtacccgccggaagcgcgtcgtatttccgcgtacctggaagcacgtccgaacccgttctctgactctgtactgttcttcggtctgcagacctacctgaaagacgttctgctgaaaccgatcaccgcaagcgatatcgcagctgcggatcgtatttgtgcggcacacggtgttccattcaatcgcgaaggctgggagcagatcctgactgatcacggtggtctgttcccactggaaatcaaagcgctgccggaaggcactctggcaccatctggtgtacctctggtgcaggtagaaaacaccgatgaacgtatgccgtggctgaccacctgggtggaaactgctctgctgcgttctgtatggtacccgtccactgtagctaccctgagcttcaaatgtaaagaaattctgtatcgtggcctgctggatacgagcgatgatccggattctcagattccatttaagctgcacgactttggtgcgcgtggtgtttcctccgcggaatccgctgcactgggtggtatggcacatctggtaaactttgccggcaccgacacgatggaagctctggaagcggcaatgacctggtatggtgctgatgtagccggtttctccattccggcagcagaacactccaccatgacttcttggggtcgtgaacgtgaggttgatgcgtatcgcaacatgctggttcagttcggtcgcccgaacgctccggttgctgttgtatctgactcctacgatctgggtaacgctgttgaaaacctgtggtgcggccgtctgaaagacgaagtgctgaaatctggtgcaacggtcgtcatccgtccagattctggcgacccggttgaaatgccactgaaagtgatggaaaccctgtggcagcactacggcggcagcgaaaactccaaaggtgcacgtgtgctgcatccttctgtccgtgtgatccagggtgacggcatgaagctggataccatccgccagctggtcgaagagctggtacgtcgcaactggtctgttgacaacattgcagtaggtatgggcggcggtctgctgcaacaggtgaaccgtgataccatgcgcttcgctatgaaagcaaacgcgatgaaaaccgctgacggcacctggcacgatgtttccaaaaacccggctaccgatcctggtaaggcttctaaagcaggccgtcaagccactgtgctggaaaacggcgtactgtccgcggttcgcctggaagcagttggcggtcgtactgatcagctgcagacggtctaccgtaacggtgttctggtaaaggactggaccttcgaagaagttcgcgcactggcgcgcaaacacctgctggaacgcgttgcttct

SEQ ID NO: 23 - protein, 482 aa, Luteibacter
MLWVMTTHSVSYLDNPILDTDSYKASHWLQYPPNTDATFFYVESRGGTYDRTLFFGLQAVLKARLERPVTHADVDEARDFFAAHGEPFNDEGWRYIVDTHGGRLPVRVRAVPEGSVVPTHQALVTIESTDPRTYWLPSYLETRLLRLWYPVTVATTSWHARQTIAHYLDTTSDDPAAQIPFKLHDFGARGVSSAESAGLGGMAHLVNFLGTDTVSGVLAARAYYGEPMAGFSIPAAEHSTITSWGRDHEVDAYRNMLRHFAKPGSLVAVVSDSYDIYHAIKEHWGKTLRDEVIASGATVVVRPDSGDPVEVVHRCVSLLDEAFGSTVNGKGYRVLNHVRVIQGDGVNPDSIRAILERITTAGYSADNLAFGMGGALLQKLTRDTQKFALKCSAARVDGAWRDVWKDPVTDQGKLSKRGRMTLLHHRESGTYRTVPLPGDAIAMPPEAIEPGWEEAMVTVWENGEPVREWSFADVRERAAAGG

SEQ ID NO: 24 - DNA, 1446 bp, Luteibacter sp.
atgctgtgggttatgaccacccactctgtttcttacctggacaacccgatcctggacaccgactcttacaaagcttctcactggctgcagtacccgccgaacaccgacgctaccttcttctacgttgaatctcgtggtggtacctacgaccgtaccctgttcttcggtctgcaggctgttctgaaagctcgtctggaacgtccggttacccacgctgacgttgacgaagctcgtgacttcttcgctgctcacggtgaaccgttcaacgacgaaggttggcgttacatcgttgacacccacggtggtcgtctgccggttcgtgttcgtgctgttccggaaggttctgttgttccgacccaccaggctctggttaccatcgaatctaccgacccgcgtacctactggctgccgtcttacctggaaacccgtctgctgcgtctgtggtacccggttaccgttgctaccacctcttggcacgctcgtcagaccatcgctcactacctggacaccacctctgacgacccggctgctcagatcccgttcaaactgcacgacttcggtgctcgtggtgtttcttctgctgaatctgctggtctgggtggtatggctcacctggttaacttcctgggtaccgacaccgtttctggtgttctggctgctcgtgcttactacggtgaaccgatggctggtttctctatcccggctgctgaacactctaccatcacctcttggggtcgtgaccacgaagttgacgcttaccgtaacatgctgcgtcacttcgctaaaccgggttctctggttgctgttgtttctgactcttacgacatctaccacgctatcaaagaacactggggtaaaaccctgcgtgacgaagttatcgcttctggtgctaccgttgttgttcgtccggactctggtgacccggttgaagttgttcaccgttgcgtttctctgctggacgaagctttcggttctaccgttaacggtaaaggttaccgtgttctgaaccacgttcgtgttatccagggtgacggtgttaacccggactctatccgtgctatcctggaacgtatcaccaccgctggttactctgctgacaacctggctttcggtatgggtggtgctctgctgcagaaactgacccgtgacacccagaaattcgctctgaaatgctctgctgctcgtgttgacggtgcttggcgtgacgtttggaaagacccggttaccgaccagggtaaactgtctaaacgtggtcgtatgaccctgctgcaccaccgtgaatctggtacctaccgtaccgttccgctgccgggtgacgctatcgctatgccgccggaagctatcgaaccgggttgggaagaagctatggttaccgtttgggaaaacggtgaaccggttcgtgaatggtctttcgctgacgttcgtgaacgtgctgctgctggtggt

SEQ ID NO: 25 - DNA, 39 bp, Artificial Sequence
  primer (Nampt_S247X-F)
  misc_feature (15)..(16): n is a, c, g, or t
ccagcatcccggcannsgaacatagcgttatgtcgagcc

SEQ ID NO: 26 - DNA, 13 bp, Artificial Sequence
  primer (Nampt_S247X-R)
gccgggatgctgg

SEQ ID NO: 27 - DNA, 27 bp, Artificial Sequence
  primer (Nampt_E248X-F)
  misc_feature (7)..(8): n is a, c, g, or t
gcatcgnnscatagcgttatgtcgagc

SEQ ID NO: 28 - DNA, 27 bp, Artificial Sequence
  primer (Nampt_E248X-R)
  misc_feature (8)..(9): n is a, c, g, or t
gctatgsnncgatgccgggatgctggt

SEQ ID NO: 29 - DNA, 36 bp, Artificial Sequence
  primer (Nampt_S253X-F)
  misc_feature (21)..(22): n is a, c, g, or t
catcggaacatagcgttatgnnsagccacggcgtcg

SEQ ID NO: 30 - DNA, 20 bp, Artificial Sequence
  primer (Nampt_S253X-R)
cataacgctatgttccgatg

SEQ ID NO: 31 - DNA, 46 bp, Artificial Sequence
  primer (Nampt_V278X-F)
  misc_feature (23)..(24): n is a, c, g, or t
cccgcataacatgctgtctattnnsagtgataccacggacttttgg

SEQ ID NO: 32 - DNA, 22 bp, Artificial Sequence
  primer (Nampt_V278X-R)
aatagacagcatgttatgcggg

SEQ ID NO: 33 - DNA, 43 bp, Artificial Sequence
  primer (Nampt_T281X-F)
  misc_feature (23)..(24): n is a, c, g, or t
catgctgtctattgtcagtgatnnsacggacttttggcacaac

SEQ ID NO: 34 - DNA, 22 bp, Artificial Sequence
  primer (Nampt_T281X-R)
atcactgacaatagacagcatg

SEQ ID NO: 35 - DNA, 20 bp, Artificial Sequence
  primer (T7-PP)
taatacgactcactataggg

SEQ ID NO: 36 - DNA, 20 bp, Artificial Sequence
  primer (T7-TP)
atgctagttattgctcagcg

SEQ ID NO: 37 - DNA, 39 bp, Artificial Sequence
  primer (Nampt_S247Z-F)
ccagcatcccggcawcygaacatagcgttatgtcgagcc

SEQ ID NO: 38 - DNA, 13 bp, Artificial Sequence
  primer (Nampt_S247Z-R)
gccgggatgctgg

SEQ ID NO: 39 - DNA, 36 bp, Artificial Sequence
  primer (Nampt_S253U-F)
catcggaacatagcgttatgrstagccacggcgtcg

SEQ ID NO: 40 - DNA, 20 bp, Artificial Sequence
  primer (Nampt_S253U-R)
cataacgctatgttccgatg

SEQ ID NO: 41 - DNA, 51 bp, Artificial Sequence
  primer (Nampt_V278J_T281B-F)
ccgcataacatgctgtctattgyyagtgatwcyacggacttttggcacaac

SEQ ID NO: 42 - DNA, 67 bp, Artificial Sequence
  primer (Nampt_V278J_T281B-R)
gacagcatgttatgcgggaatttagccatcagatagcgaaacgtgctcagttcatcgacgccgtggc

SEQ ID NO: 43 - DNA, 28 bp, Artificial Sequence
  primer (MrNampt_M230T-F)
tccggcgaccgaacacagcaccgttacc

SEQ ID NO: 44 - DNA, 27 bp, Artificial Sequence
  primer (MrNampt_M230T-R)
tgtgttcggtcgccggaatgctatagc

SEQ ID NO: 45 - DNA, 27 bp, Artificial Sequence
  primer (MrNampt_E231G-F)
ggcgatgggccacagcaccgttaccag

SEQ ID NO: 46 - DNA, 29 bp, Artificial Sequence
  primer (MrNampt_E231G-R)
gtgctgtggcccatcgccggaatgctata

SEQ ID NO: 47 - DNA, 29 bp, Artificial Sequence
  primer (MrNampt_V264A-F)
ggcgatggcgatcgacagctataaccgtg

SEQ ID NO: 48 - DNA, 27 bp, Artificial Sequence
  primer (MrNampt_V264A-R)
tgtcgatcgccatcgccatcagcgcac

SEQ ID NO: 49 - DNA, 27 bp, Artificial Sequence
  primer (SpNampt_E227G-F)
ggcagcaggccatagcaccatgaccag

SEQ ID NO: 50 - DNA, 28 bp, Artificial Sequence
  primer (SpNampt_E227G-R)
tgctatggcctgctgccggaatgctaaa